European Patent Application EP 4 238 995 A1, published September 6, 2023. Title: WARS Neutralizing Antibodies and Uses Thereof. Applicant: MirimGENE Co., Ltd. The sequence listing filed with the application follows.

SEQUENCE LISTING (26 sequences)

SEQ ID NO: 1 - protein, 121 aa, Artificial Sequence
  GKB101 - VH
EVQLLESGGGLVQPGGSLRLSCAASGFTFSSYDMSWVRQAPGKGLEWVSAISSGGSSIYYADSVKGRFTISRDNSKNTLYLQMNSLRAEDTAVYYCARDVAWDMLGDFDYWGQGTLVTVSS

SEQ ID NO: 2 - protein, 109 aa, Artificial Sequence
  GKB101 - VL
QSVLTQPPSASGTPGQRVTISCTGSSSNIGSNYVYWYQQLPGTAPKLLIYANSHRPSGVPDRFSGSKSGTSASLAISGLRSEDEADYYCGAWDDSLSAYVFGGGTKLTV

SEQ ID NO: 3 - protein, 5 aa, Artificial Sequence
  GKB101 - VH CDR1
SYDMS

SEQ ID NO: 4 - protein, 17 aa, Artificial Sequence
  GKB101 - VH CDR2
AISSGGSSIYYADSVKG

SEQ ID NO: 5 - protein, 12 aa, Artificial Sequence
  GKB101 - VH CDR3
DVAWDMLGDFDY

SEQ ID NO: 6 - protein, 11 aa, Artificial Sequence
  GKB101 - VL CDR1
SSSNIGSNYVY

SEQ ID NO: 7 - protein, 7 aa, Artificial Sequence
  GKB101 - VL CDR2
ANSHRPS

SEQ ID NO: 8 - protein, 9 aa, Artificial Sequence
  GKB101 - VL CDR3
GAWDDSLSA

SEQ ID NO: 9 - DNA, 51 bp, Artificial Sequence
  CDR_primer_F
gtggccacagcggccgatgtccactcggaagtacagttggtcgaaagtggc

SEQ ID NO: 10 - DNA, 51 bp, Artificial Sequence
  CDR_primer_R
gaagaccgatgggcccttggtgctagccgatgagacggtcactaaagtgcc

SEQ ID NO: 11 - DNA, 50 bp, Artificial Sequence
  VL_primer_F
gccacagcggccgatgtccactcggacattcaaatgacgcagagtccctc

SEQ ID NO: 12 - DNA, 53 bp, Artificial Sequence
  VL_primer_R
gaagacagatggtgcagccacagatcttttaatttccactttagttccctgcc

SEQ ID NO: 13 - DNA, 51 bp, Artificial Sequence
  CH_primer_F
ggcactttagtgaccgtctcatcggctagcaccaagggcccatcggtcttc

SEQ ID NO: 14 - DNA, 51 bp, Artificial Sequence
  CH_primer_R
gccactttcgaccaactgtacttccgagtggacatcggccgctgtggccac

SEQ ID NO: 15 - DNA, 53 bp, Artificial Sequence
  CL_primer_F
ggcagggaactaaagtggaaattaaaagatctgtggctgcaccatctgtcttc

SEQ ID NO: 16 - DNA, 50 bp, Artificial Sequence
  CL_primer_R
gagggactctgcgtcatttgaatgtccgagtggacatcggccgctgtggc

SEQ ID NO: 17 - DNA, 51 bp, Artificial Sequence
  VH1-69_Forward
gtggccacagcggccgatgtccactcgcaagttcagctggtccagagcggc

SEQ ID NO: 18 - DNA, 52 bp, Artificial Sequence
  VH1-69_Reverse
gaagaccgatgggcccttggtgctagccgatgagacggtaaccagagtaccc

SEQ ID NO: 19 - DNA, 52 bp, Artificial Sequence
  CH1-69_Forward
gccgctctggaccagctgaacttgcgagtggacatcggccgctgtggccacc

SEQ ID NO: 20 - DNA, 52 bp, Artificial Sequence
  CH1-69_Reverse
gggtactctggttaccgtctcatcggctagcaccaagggcccatcggtcttc

SEQ ID NO: 21 - protein, 106 aa, Artificial Sequence
  GKB101 - CL
TVAAPSVFIFPPSDEQLKSGTASVVCLLNNFYPREAKVQWKVDNALQSGNSQESVTEQDSKDSTYSLSSTLTLSKADYEKHKVYACEVTHQGLSSPVTKSFNRGEC

SEQ ID NO: 22 - protein, 98 aa, Artificial Sequence
  GKB101 - CH1
ASTKGPSVFPLAPSSKSTSGGTAALGCLVKDYFPEPVTVSWNSGALTSGVHTFPAVLQSSGLYSLSSVVTVPSSSLGTQTYICNVNHKPSNTKVDKKV

SEQ ID NO: 23 - protein, 23 aa, Artificial Sequence
  GKB101 - Hinge
EPKSCDKTHTCPPCPAPELLGGP

SEQ ID NO: 24 - protein, 103 aa, Artificial Sequence
  GKB101 - CH2
SVFLFPPKPKDTLMISRTPEVTCVVVDVSHEDPEVKFNWYVDGVEVHNAKTKPREEQYNSTYRVVSVLTVLHQDWLNGKEYKCKVSNKALPAPIEKTISKAKG

SEQ ID NO: 25 - protein, 100 aa, Artificial Sequence
  GKB101 - CH3
REPQVYTLPPSREEMTKNQVSLTCLVKGFYPSDIAVEWESNGQPENNYKTTPPVLDSDGSFFLYSKLTVDKSRWQQGNVFSCSVMHEALHNHYTQKSLSL

SEQ ID NO: 26 - protein, 471 aa, Artificial Sequence
  WARS
MPNSEPASLLELFNSIATQGELVRSLKAGNASKDEIDSAVKMLVSLKMSYKAAAGEDYKADCPPGNPAPTSNHGPDATEAEEDFVDPWTVQTSSAKGIDYDKLIVRFGSSKIDKELINRIERATGQRPHHFLRRGIFFSHRDMNQVLDAYENKKPFYLYTGRGPSSEAMHVGHLIPFIFTKWLQDVFNVPLVIQMTDDEKYLWKDLTLDQAYSYAVENAKDIIACGFDINKTFIFSDLDYMGMSSGFYKNVVKIQKHVTFNQVKGIFGFTDSDCIGKISFPAIQAAPSFSNSFPQIFRDRTDIQCLIPCAIDQDPYFRMTRDVAPRIGYPKPALLHSTFFPALQGAQTKMSASDPNSSIFLTDTAKQIKTKVNKHAFSGGRDTIEEHRQFGGNCDVDVSFMYLTFFLEDDDKLEQIRKDYTSGAMLTGELKKALIEVLQPLIAEHQARRKEVTDEIVKEFMTPRKLSFDFQ